European Patent Specification EP 3 689 363 B1, published September 9, 2026. Title: PHARMACEUTICAL COMPOSITION FOR PREVENTING OR TREATING CARDIAC ARRHYTHMIAS. Applicant: BethphaGen Inc. The sequence listing filed with the application follows.

SEQUENCE LISTING (42 sequences)

SEQ ID NO: 1 - protein, 250 aa, Homo sapiens
MRGTPKTHLLAFSLLCLLSKVRTQLCPTPCTCPWPPPRCPLGVPLVLDGCGCCRVCARRLGEPCDQLHVCDASQGLVCQPGAGPGGRGALCLLAEDDSSCEVNGRLYREGETFQPHCSIRCRCEDGGFTCVPLCSEDVRLPSWDCPHPRRVEVLGKCCPEWVCGQGGGLGTQPLPAQGPQFSGLVSSLPPGVPCPEWSTAWGPCSTTCGLGMATRVSNQNRFCRLETQRRLCLSRPCPPSRGRSPQNSAF

SEQ ID NO: 2 - DNA, 750 bp, Homo sapiens
atgagaggcacaccgaagacccacctcctggccttctccctcctctgcctcctctcaaaggtgcgtacccagctgtgcccgacaccatgtacctgcccctggccacctccccgatgcccgctgggagtacccctggtgctggatggctgtggctgctgccgggtatgtgcacggcggctgggggagccctgcgaccaactccacgtctgcgacgccagccagggcctggtctgccagcccggggcaggacccggtggccggggggccctgtgcctcttggcagaggacgacagcagctgtgaggtgaacggccgcctgtatcgggaaggggagaccttccagccccactgcagcatccgctgccgctgcgaggacggcggcttcacctgcgtgccgctgtgcagcgaggatgtgcggctgcccagctgggactgcccccaccccaggagggtcgaggtcctgggcaagtgctgccctgagtgggtgtgcggccaaggagggggactggggacccagccccttccagcccaaggaccccagttttctggccttgtctcttccctgccccctggtgtcccctgcccagaatggagcacggcctggggaccctgctcgaccacctgtgggctgggcatggccacccgggtgtccaaccagaaccgcttctgccgactggagacccagcgccgcctgtgcctgtccaggccctgcccaccctccaggggtcgcagtccacaaaacagtgccttc

SEQ ID NO: 3 - protein, 997 aa, Homo sapiens
MENAHTKTVEEVLGHFGVNESTGLSLEQVKKLKERWGSNELPAEEGKTLLELVIEQFEDLLVRILLLAACISFVLAWFEEGEETITAFVEPFVILLILVANAIVGVWQERNAENAIEALKEYEPEMGKVYRQDRKSVQRIKAKDIVPGDIVEIAVGDKVPADIRLTSIKSTTLRVDQSILTGESVSVIKHTDPVPDPRAVNQDKKNMLFSGTNIAAGKAMGVVVATGVNTEIGKIRDEMVATEQERTPLQQKLDEFGEQLSKVISLICIAVWIINIGHFNDPVHGGSWIRGAIYYFKIAVALAVAAIPEGLPAVITTCLALGTRRMAKKNAIVRSLPSVETLGCTSVICSDKTGTLTTNQMSVCRMFILDRVEGDTCSLNEFTITGSTYAPIGEVHKDDKPVNCHQYDGLVELATICALCNDSALDYNEAKGVYEKVGEATETALTCLVEKMNVFDTELKGLSKIERANACNSVIKQLMKKEFTLEFSRDRKSMSVYCTPNKPSRTSMSKMFVKGAPEGVIDRCTHIRVGSTKVPMTSGVKQKIMSVIREWGSGSDTLRCLALATHDNPLRREEMHLEDSANFIKYETNLTFVGCVGMLDPPRIEVASSVKLCRQAGIRVIMITGDNKGTAVAICRRIGIFGQDEDVTSKAFTGREFDELNPSAQRDACLNARCFARVEPSHKSKIVEFLQSFDEITAMTGDGVNDAPALKKAEIGIAMGSGTAVAKTASEMVLADDNFSTIVAAVEEGRAIYNNMKQFIRYLISSNVGEVVCIFLTAALGFPEALIPVQLLWVNLVTDGLPATALGFNPPDLDIMNKPPRNPKEPLISGWLFFRYLAIGCYVGAATVGAAAWWFIAADGGPRVSFYQLSHFLQCKEDNPDFEGVDCAIFESPYPMTMALSVLVTIEMCNALNSLSENQSLLRMPPWENIWLVGSICLSMSLHFLILYVEPLPLIFQITPLNVTQWLMVLKISLPVILMDETLKFVARNYLEPAILE

SEQ ID NO: 4 - DNA, 2991 bp, Homo sapiens
atggagaacgcgcacaccaagacggtggaggaggtgctgggccacttcggcgtcaacgagagtacggggctgagcctggaacaggtcaagaagcttaaggagagatggggctccaacgagttaccggctgaagaaggaaaaaccttgctggaacttgtgattgagcagtttgaagacttgctagttaggattttattactggcagcatgtatatcttttgttttggcttggtttgaagaaggtgaagaaacaattacagcctttgtagaaccttttgtaattttactcatattagtagccaatgcaattgtgggtgtatggcaggaaagaaatgctgaaaatgccatcgaagcccttaaggaatatgagcctgaaatgggcaaagtgtatcgacaggacagaaagagtgtgcagcggattaaagctaaagacatagttcctggtgatattgtagaaattgctgttggtgacaaagttcctgctgatataaggttaacttccatcaaatctaccacactaagagttgaccagtcaattctcacaggtgaatctgtctctgtcatcaagcacactgatcccgtccctgacccacgagctgtcaaccaagataaaaagaacatgctgttttctggtacaaacattgctgctgggaaagctatgggagtggtggtagcaactggagttaacaccgaaattggcaagatccgggatgaaatggtggcaacagaacaggagagaacaccccttcagcaaaaactagatgaatttggggaacagctttccaaagtcatctcccttatttgcattgcagtctggatcataaatattgggcacttcaatgacccggttcatggagggtcctggatcagaggtgctatttactactttaaaattgcagtggccctggctgtagcagccattcctgaaggtctgcctgcagtcatcaccacctgcctggctcttggaactcgcagaatggcaaagaaaaatgccattgttcgaagcctcccgtctgtggaaacccttggttgtacttctgttatctgctcagacaagactggtacacttacaacaaaccagatgtcagtctgcaggatgttcattctggacagagtggaaggtgatacttgttcccttaatgagtttaccataactggatcaacttatgcacctattggagaagtgcataaagatgataaaccagtgaattgtcaccagtatgatggtctggtagaattagcaacaatttgtgctctttgtaatgactctgctttggattacaatgaggcaaagggtgtgtatgaaaaagttggagaagctacagagactgctctcacttgcctagtagagaagatgaatgtatttgataccgaattgaagggtctttctaaaatagaacgtgcaaatgcctgcaactcagtcattaaacagctgatgaaaaaggaattcactctagagttttcacgtgacagaaagtcaatgtcggtttactgtacaccaaataaaccaagcaggacatcaatgagcaagatgtttgtgaagggtgctcctgaaggtgtcattgacaggtgcacccacattcgagttggaagtactaaggttcctatgacctctggagtcaaacagaagatcatgtctgtcattcgagagtggggtagtggcagcgacacactgcgatgcctggccctggccactcatgacaacccactgagaagagaagaaatgcaccttgaggactctgccaactttattaaatatgagaccaatctgaccttcgttggctgcgtgggcatgctggatcctccgagaatcgaggtggcctcctccgtgaagctgtgccggcaagcaggcatccgggtcatcatgatcactggggacaacaagggcactgctgtggccatctgtcgccgcatcggcatcttcgggcaggatgaggacgtgacgtcaaaagctttcacaggccgggagtttgatgaactcaacccctccgcccagcgagacgcctgcctgaacgcccgctgttttgctcgagttgaaccctcccacaagtctaaaatcgtagaatttcttcagtcttttgatgagattacagctatgactggcgatggcgtgaacgatgctcctgctctgaagaaagccgagattggcattgctatgggctctggcactgcggtggctaaaaccgcctctgagatggtcctggcggatgacaacttctccaccattgtggctgccgttgaggaggggcgggcaatctacaacaacatgaaacagttcatccgctacctcatctcgtccaacgtcggggaagttgtctgtattttcctgacagcagcccttggatttcccgaggctttgattcctgttcagctgctctgggtcaatctggtgacagatggcctgcctgccactgcactggggttcaaccctcctgatctggacatcatgaataaacctccccggaacccaaaggaaccattgatcagcgggtggctctttttccgttacttggctattggctgttacgtcggcgctgctaccgtgggtgctgctgcatggtggttcattgctgctgacggtggtccaagagtgtccttctaccagctgagtcatttcctacagtgtaaagaggacaacccggactttgaaggcgtggattgtgcaatctttgaatccccatacccgatgacaatggcgctctctgttctagtaactatagaaatgtgtaacgccctcaacagcttgtccgaaaaccagtccttgctgaggatgcccccctgggagaacatctggctcgtgggctccatctgcctgtccatgtcactccacttcctgatcctctatgtcgaacccttgccactcatcttccagatcacaccgctgaacgtgacccagtggctgatggtgctgaaaatctccttgcccgtgattctcatggatgagacgctcaagtttgtggcccgcaactacctggaacctgcaatactggag

SEQ ID NO: 5 - protein, 22 aa, Artificial Sequence
  self-cleavage sequence derived from porcine teschovirus-1
GSGATNFSLLKQAGDVEENPGP

SEQ ID NO: 6 - DNA, 66 bp, Artificial Sequence
  self-cleavage sequence derived from porcine teschovirus-1
ggaagcggagctactaacttcagcctgctgaagcaggctggagacgtggaggagaaccctggacct

SEQ ID NO: 7 - protein, 21 aa, Artificial Sequence
  self-cleavage sequence derived from Thoseaasigna virus
GSGEGRGSLLTCGDVEENPGP

SEQ ID NO: 8 - DNA, 63 bp, Artificial Sequence
  self-cleavage sequence derived from Thoseaasigna virus
ggaagcggagagggcagaggaagtctgctaacatgcggtgacgtcgaggagaatcctggacct

SEQ ID NO: 9 - protein, 23 aa, Artificial Sequence
  self-cleavage sequence derived from equine rhinitis A virus (ERAV)
GSGQCTNYALLKLAGDVESNPGP

SEQ ID NO: 10 - DNA, 69 bp, Artificial Sequence
  self-cleavage sequence derived from equine rhinitis A virus (ERAV)
ggaagcggacagtgtactaattatgctctcttgaaattggctggagatgttgagagcaaccctggacct

SEQ ID NO: 11 - protein, 25 aa, Artificial Sequence
  self-cleavage sequence derived from FMDV 2A
GSGVKQTLNFDLLKLAGDVESNPGP

SEQ ID NO: 12 - DNA, 75 bp, Artificial Sequence
  self-cleavage sequence derived from FMDV 2A
ggaagcggagtgaaacagactttgaattttgaccttctcaagttggcgggagacgtggagtccaaccctggacct

SEQ ID NO: 13 - DNA, 18 bp, Artificial Sequence
  Forward primer for Mouse alpha-SMA
cccacccagagtggagaa

SEQ ID NO: 14 - DNA, 20 bp, Artificial Sequence
  Reverse primer for Mouse alpha-SMA
acatagctggagcagcgtct

SEQ ID NO: 15 - DNA, 21 bp, Artificial Sequence
  Forward primer for Mouse Collagen I
catgttcagctttgtggacct

SEQ ID NO: 16 - DNA, 20 bp, Artificial Sequence
  Reverse primer for Mouse Collagen I
gacgctgacttcagggatgt

SEQ ID NO: 17 - DNA, 20 bp, Artificial Sequence
  Forward primer for Mouse TGF-beta 1
tggagcaacatgtggaactc

SEQ ID NO: 18 - DNA, 18 bp, Artificial Sequence
  Reverse primer for Mouse TGF-beta 1
cagcagccggttaccaag

SEQ ID NO: 19 - DNA, 24 bp, Artificial Sequence
  Forward primer for Mouse IL-1 beta
tccaggatgaggacatgatgagca

SEQ ID NO: 20 - DNA, 25 bp, Artificial Sequence
  Reverse primer for Mouse IL-1 beta
gaacgtcacacacaccagcaggtta

SEQ ID NO: 21 - DNA, 21 bp, Artificial Sequence
  Forward primer for Mouse RANTES
tgcagaggactctgagacagc

SEQ ID NO: 22 - DNA, 19 bp, Artificial Sequence
  Reverse primer for Mouse RANTES
gagtggtgtccgagccata

SEQ ID NO: 23 - DNA, 20 bp, Artificial Sequence
  Forward primer for Mouse F4/80
cctggacgaatcctgtgaag

SEQ ID NO: 24 - DNA, 20 bp, Artificial Sequence
  Reverse primer for Mouse F4/80
ggtgggaccacagagagttg

SEQ ID NO: 25 - DNA, 18 bp, Artificial Sequence
  Forward primer for Mouse MCP-1
catccacgtgttggctca

SEQ ID NO: 26 - DNA, 23 bp, Artificial Sequence
  Reverse primer for Mouse MCP-1
gatcatcttgctggtgaatgagt

SEQ ID NO: 27 - DNA, 20 bp, Artificial Sequence
  Forward primer for Mouse CCN5
atacaggtgccaggaaggtg

SEQ ID NO: 28 - DNA, 20 bp, Artificial Sequence
  Reverse primer for Mouse CCN5
gttggatactcgggtggcta

SEQ ID NO: 29 - DNA, 20 bp, Artificial Sequence
  Forward primer for Mouse GAPDH
ctcatgaccacagtccatgc

SEQ ID NO: 30 - DNA, 20 bp, Artificial Sequence
  Reverse primer for Mouse GAPDH
ttcagctctgggatgacctt

SEQ ID NO: 31 - DNA, 20 bp, Artificial Sequence
  Forward primer for Mouse 18s rRNA
gtaacccgttgaaccccatt

SEQ ID NO: 32 - DNA, 20 bp, Artificial Sequence
  Reverse primer for Mouse 18s rRNA
ccatccaatcggtagtagcg

SEQ ID NO: 33 - DNA, 27 bp, Artificial Sequence
  Forward primer for Rat alpha-SMA
tctgtctctagcacacaactgtgaatg

SEQ ID NO: 34 - DNA, 23 bp, Artificial Sequence
  Reverse primer for Rat alpha-SMA
ttgacaggccagggctagaaggg

SEQ ID NO: 35 - DNA, 26 bp, Artificial Sequence
  Forward primer for Rat Collagen I
aatgcacttttggtttttggtcacgt

SEQ ID NO: 36 - DNA, 21 bp, Artificial Sequence
  Reverse primer for Rat Collagen I
cagcccactttgccccaaccc

SEQ ID NO: 37 - DNA, 20 bp, Artificial Sequence
  Forward primer for Rat TGF-beta 1
tgttcgcgctctcggcagtg

SEQ ID NO: 38 - DNA, 20 bp, Artificial Sequence
  Reverse primer for Rat TGF-beta 1
cggatggcctcgatgcgctt

SEQ ID NO: 39 - DNA, 22 bp, Artificial Sequence
  Forward primer for Rat GAPDH
acccagcccagcaaggatactg

SEQ ID NO: 40 - DNA, 23 bp, Artificial Sequence
  Reverse primer for Rat GAPDH
attcgagagaagggagggctccc

SEQ ID NO: 41 - DNA, 753 bp, Homo sapiens
atgagaggcacaccgaagacccacctcctggccttctccctcctctgcctcctctcaaaggtgcgtacccagctgtgcccgacaccatgtacctgcccctggccacctccccgatgcccgctgggagtacccctggtgctggatggctgtggctgctgccgggtatgtgcacggcggctgggggagccctgcgaccaactccacgtctgcgacgccagccagggcctggtctgccagcccggggcaggacccggtggccggggggccctgtgcctcttggcagaggacgacagcagctgtgaggtgaacggccgcctgtatcgggaaggggagaccttccagccccactgcagcatccgctgccgctgcgaggacggcggcttcacctgcgtgccgctgtgcagcgaggatgtgcggctgcccagctgggactgcccccaccccaggagggtcgaggtcctgggcaagtgctgccctgagtgggtgtgcggccaaggagggggactggggacccagccccttccagcccaaggaccccagttttctggccttgtctcttccctgccccctggtgtcccctgcccagaatggagcacggcctggggaccctgctcgaccacctgtgggctgggcatggccacccgggtgtccaaccagaaccgcttctgccgactggagacccagcgccgcctgtgcctgtccaggccctgcccaccctccaggggtcgcagtccacaaaacagtgccttctag

SEQ ID NO: 42 - DNA, 2994 bp, Homo sapiens
atggagaacgcgcacaccaagacggtggaggaggtgctgggccacttcggcgtcaacgagagtacggggctgagcctggaacaggtcaagaagcttaaggagagatggggctccaacgagttaccggctgaagaaggaaaaaccttgctggaacttgtgattgagcagtttgaagacttgctagttaggattttattactggcagcatgtatatcttttgttttggcttggtttgaagaaggtgaagaaacaattacagcctttgtagaaccttttgtaattttactcatattagtagccaatgcaattgtgggtgtatggcaggaaagaaatgctgaaaatgccatcgaagcccttaaggaatatgagcctgaaatgggcaaagtgtatcgacaggacagaaagagtgtgcagcggattaaagctaaagacatagttcctggtgatattgtagaaattgctgttggtgacaaagttcctgctgatataaggttaacttccatcaaatctaccacactaagagttgaccagtcaattctcacaggtgaatctgtctctgtcatcaagcacactgatcccgtccctgacccacgagctgtcaaccaagataaaaagaacatgctgttttctggtacaaacattgctgctgggaaagctatgggagtggtggtagcaactggagttaacaccgaaattggcaagatccgggatgaaatggtggcaacagaacaggagagaacaccccttcagcaaaaactagatgaatttggggaacagctttccaaagtcatctcccttatttgcattgcagtctggatcataaatattgggcacttcaatgacccggttcatggagggtcctggatcagaggtgctatttactactttaaaattgcagtggccctggctgtagcagccattcctgaaggtctgcctgcagtcatcaccacctgcctggctcttggaactcgcagaatggcaaagaaaaatgccattgttcgaagcctcccgtctgtggaaacccttggttgtacttctgttatctgctcagacaagactggtacacttacaacaaaccagatgtcagtctgcaggatgttcattctggacagagtggaaggtgatacttgttcccttaatgagtttaccataactggatcaacttatgcacctattggagaagtgcataaagatgataaaccagtgaattgtcaccagtatgatggtctggtagaattagcaacaatttgtgctctttgtaatgactctgctttggattacaatgaggcaaagggtgtgtatgaaaaagttggagaagctacagagactgctctcacttgcctagtagagaagatgaatgtatttgataccgaattgaagggtctttctaaaatagaacgtgcaaatgcctgcaactcagtcattaaacagctgatgaaaaaggaattcactctagagttttcacgtgacagaaagtcaatgtcggtttactgtacaccaaataaaccaagcaggacatcaatgagcaagatgtttgtgaagggtgctcctgaaggtgtcattgacaggtgcacccacattcgagttggaagtactaaggttcctatgacctctggagtcaaacagaagatcatgtctgtcattcgagagtggggtagtggcagcgacacactgcgatgcctggccctggccactcatgacaacccactgagaagagaagaaatgcaccttgaggactctgccaactttattaaatatgagaccaatctgaccttcgttggctgcgtgggcatgctggatcctccgagaatcgaggtggcctcctccgtgaagctgtgccggcaagcaggcatccgggtcatcatgatcactggggacaacaagggcactgctgtggccatctgtcgccgcatcggcatcttcgggcaggatgaggacgtgacgtcaaaagctttcacaggccgggagtttgatgaactcaacccctccgcccagcgagacgcctgcctgaacgcccgctgttttgctcgagttgaaccctcccacaagtctaaaatcgtagaatttcttcagtcttttgatgagattacagctatgactggcgatggcgtgaacgatgctcctgctctgaagaaagccgagattggcattgctatgggctctggcactgcggtggctaaaaccgcctctgagatggtcctggcggatgacaacttctccaccattgtggctgccgttgaggaggggcgggcaatctacaacaacatgaaacagttcatccgctacctcatctcgtccaacgtcggggaagttgtctgtattttcctgacagcagcccttggatttcccgaggctttgattcctgttcagctgctctgggtcaatctggtgacagatggcctgcctgccactgcactggggttcaaccctcctgatctggacatcatgaataaacctccccggaacccaaaggaaccattgatcagcgggtggctctttttccgttacttggctattggctgttacgtcggcgctgctaccgtgggtgctgctgcatggtggttcattgctgctgacggtggtccaagagtgtccttctaccagctgagtcatttcctacagtgtaaagaggacaacccggactttgaaggcgtggattgtgcaatctttgaatccccatacccgatgacaatggcgctctctgttctagtaactatagaaatgtgtaacgccctcaacagcttgtccgaaaaccagtccttgctgaggatgcccccctgggagaacatctggctcgtgggctccatctgcctgtccatgtcactccacttcctgatcctctatgtcgaacccttgccactcatcttccagatcacaccgctgaacgtgacccagtggctgatggtgctgaaaatctccttgcccgtgattctcatggatgagacgctcaagtttgtggcccgcaactacctggaacctgcaatactggagtag